European Patent Specification EP 3 874 032 B1, published April 1, 2026. Title: Enzymatic Production of Hexoses. Applicant: Bonumose LLC. The sequence listing filed with the application follows.

SEQUENCE LISTING (26 sequences)

SEQ ID NO: 1 - protein, 456 aa, Thermococcus kodakaraensis
MGKLFGTFGVRGIANEEITPEFALKIGMAFGTLLKREGRERPLVVVGRDTRVSGEMLKDALISGLLSTGCDVIDVGIAPTPAIQWATNHFNADGGAVITASHNPPEYNGIKLLEPNGMGLKKEREAIVEELFFSEDFHRAKWNEIGELRKEDIIKPYIEAIKNRVDVEAIKKRRPFVVVDTSNGAGSLTLPYLLRELGCKVVSVNAHPDGHFPARNPEPNEENLKGFMEIVKALGADFGVAQDGDADRAVFIDENGRFIQGDKTFALVADAVLRENGGGLLVTTIATSNLLDDIAKRNGAKVMRTKVGDLIVARALLENNGTIGGEENGGVIFPDFVLGRDGAMTTAKIVEIFAKSGKKFSELIDELPKYYQFKTKRHVEGDRKAIVAKVAELAEKKGYKIDTTDGTKIIFDDGWVLVRASGTEPIIRIFSEAKSEEKAREYLELGIKLLEEALKG

SEQ ID NO: 2 - protein, 582 aa, Geobacillus stearothermophilus NUB3621
MDWKSKYEQWLAYKPLDEELKQLLQKRQDDWKWLEDGFYKNLEFGTGGMRGEIGPGTNRMNIYTVRKASEGLARYIGSFGEEAKKRGVVIAYDSRHKSREFAMEAAKTLATHGIQTYVFDELRPTPELSFAVRYLHAFSGIVITASHNPPEYNGYKVYGEDGGQLPPETADAVIRYVNEVENELDIHVEDEAILKEKGLIQIIGEEVDNAYIEAVKTVSLQPKLAEEVDINIVFTPLHGTSNKPVRRALKELGYRNVFVVKEQEQPDPNFSTVASPNPEEHAAFALAIELGKQVNADLLIATDPDADRLGIAVKNEQGEYIVLTGNQTGGLLLYYLLSQKKEKGILPENGVVLKTIVTSEFGRVIAQSFGLDTVDTLTGFKFIGEKIKEYEQTGQYTFQFGYEESYGYLIGDFARDKDAVQAAVLAAEVCAFYKKQGMSLYEGLIQLFDQYGYYREGQQSLTLKGKEGAETIQAILTSFRNEPPTEVAGKKVTVIEDYKTKERIHTLTGEKTVITLPTSNVLKYVLEDDSWFCLRPSGTEPKIKVYFGVKGQSLADSEAKLQQLSDAVMKRVHDFLRTASLS

SEQ ID NO: 3 - protein, 581 aa, Caldibacillus debilis
MEWKQRAERWLRFENLDPELKKQLEEMAKDEKKLEDLFYKYLEFGTGGMRGEIGPGTNRINIYTVRKASEGLARFLLASGGEEKAKQGVVIAYDSRRKSREFALETAKTVGKHGIKAYVFESLRPTPELSFAVRYLHAAAGVVITASHNPPEYNGYKVYGEDGGQLTPKAADELIRYVYEVEDELSLTVPGEQELIDRGLLQYIGENIDLAYIEKLKTIQLNRDVILNGGKDLKIVFTPLHGTAGQLVQTGLREFGFQNVYVVKEQEQPDPDFSTVKSPNPEEHEAFEIAIRYGKKYDADLIMGTDPDSDRLGIVVKNGQGDYVVLTGNQTGAILLYYLLSQKKEKGMLVRNSAVLKTIVTSELGRAIASDFGVETIDTLTGFKFIGEKIKEFKETGSHVFQFGYEESYGYLIGDFVRDKDAIQAALFAAEAAAYYKAQGKSLYDVLMEIYKKYGFYKESLRSITLKGKDGAEKIRAIMDAFRQNPPEEVSGIPVAITEDYLTQKRVDKAAGQTTPIHLPKSNVLKYYLADESWFCIRPSGTEPKCKFYFAVRGDSEAQSEARLRQLETNVMAMVEKILQK

SEQ ID NO: 4 - protein, 584 aa, Geobacillus thermoglucosidasius
MDWKKKYEQWLAYEPLDEELKHSLKKHQHDLPWLEDCFYKNLEFGTGGMRGEIGPGTNRMNVYTIRKASEGLARYIESFGEDAKRRGVVIAYDSRHKSREFAMETAKTLATHGIQTYVFDELRPTPELSFAVRYLRAFSGVVITASHNPPEYNGYKVYGEDGGQLPPETADAVIRYVNEVENELEIDVEEEAVLKEKGLIQMIGEEVDNAYIDAVKTISFQPKLAEETDVNIVFTPLHGTSNKPIRRALTELGYRHVFVVEEQEHPDPNFSTVSSPNPEEHAAFALAIELGKKVNADLLIATDPDADRLGIAVKNDKGDYIVLTGNQTGGLLLHYLLSQKKEKGILPENGVVLKTIVTSEFGRAIAQSFGLDTVDTLTGFKFIGEKIKEYEQTGQYTFQFGYEESYGYLIGDFVRDKDAVQAAVLAAEVCAFYKKHGMSLYEGLLRLFDQYGYYREGQQSLTLKGKKGSETIQAILTSFRHEPPTEVAGKKVIVIEDYKTKERVNTATGEKTLIALPTSDVLKYVLEDDSWFCLRPSGTEPKLKVYFGVKGESLSDSEAKLQQLSDTVMERVRGFLNTASPFQP

SEQ ID NO: 5 - protein, 582 aa, Parageobacillus caldoxylosilyticus NBRC 107762
MDWKSKYEQWMAYEQLDGELKRLLQDRQDDLKWVEDGFYKNLEFGTGGMRGEIGPGTNRMNIYTVRKASEGLARYIESFGEEAKKRGVVIAYDSRHKSRDFAMEAAKTLATHGIQTYVFDELRPTPELSFAVRYLQAFSGIVITASHNPPEYNGYKVYGEDGGQLPPDTADAVIRYVNEVANELDIHVEDEAILKEKGLIQIIGEEVDNAYIDAVKTISLQPKLAEEVDINIVFTPLHGTSNKPVRRALKELGYRNVFVVKEQEQPDPNFSTVASPNPEEHAAFALAIELGKKVNADLLIATDPDADRLGVAVKNDQGEYVVLTGNQTGALLLHYLLSQRKEKEILPENGVVLKTIVTSEFGRAIAQSFGLETVDTLTGFKFIGEKIKEYEQTGQYTFQFGYEESYGYLIGDFVRDKDAVQAAVLAAEVCAFYKKQGMSLYEGLIHLFDRYGYYREGQQSLTLKGKEGAETIQAILTSFRNEPPTEVDGKRVTVIEDYKTKERIHTLTGEKTVITLPTSNVLKYVLEDDSWFCLRPSGTEPKIKVYFGVKGKSLADSEEKLNRLSNEVMKRVHDLLRTASLS

SEQ ID NO: 6 - protein, 567 aa, Thermobrachium celere DSM 8682
MEYMSMYKRWLEFDEETRRELEGLDEKEIMERFYKELEFGTGGLRGIIGAGTNRMNVYTVRKATQGLANFILKQNIENPSVAIAYDSRKYSDVFAKEAALVLNASGIKTYIYDELKPTPMLSYAVRHMKATAGIVITASHNPKEYNGYKVYWSDGGQVTEELAEGILNEIKNVDYSDIKRMDYDEAIEKGLFNFMPKEVEDTYVKLVKGLTVNKELVEKMKDKVKVIYTPLHGTGNKPVRRVLEELGYKNVYVVKEQENPDPAFSTVKYPNPEESEVFTRAMEMARELDADVIIGTDPDCDRVGVVVKNSEGNYVVLTGNQTGALLTHYMLENLKATNTIPKNPVVIKTIVTTEFARAICKDYGVEILDVLTGFKYIGEKIKEFEINGDMNFILGFEESYGYLAGTFVRDKDAVIASMLIVEMVCYYKDRGMSLYEGLMELYNKYGFYKEDLVSITLKGIEGSEKIKKIMEDLRSNPPKKVADLSVKLVKDYKMSVTKNVVSGEEEVIELPKSNVIQLVLEDGSVITARPSGTEPKIKFYFMTKGETLEKAEENIKRFKEEILKMAE

SEQ ID NO: 7 - protein, 473 aa, Anaerolinea thermophila
MSHTIRFGTDGWRGVIAEDYTFANVRCATQGYASYMIRHGKAGATFVIGHDKRFHSENFALAAAEVMAGNGLKVLLTDGATPTPVIAFSVVHHKAAGAINITASHNPPTDNGFKVRNEFGGAIDPEGLKEIESLIPEDESEVKRMPASEAEAKGLIQRFDPAPAYIEHLKELIDVEPIKQAGLKIVVDCMWGNGAGWFPRILSGGKTEIIEIHNERNPIFPEMKRPEPIPPNINVGLKKTVDSGADVLLITDGDADRVGVGDEKGNFINQLQVYALLALYLLEVRGERGAIVKTLSTTSMLEKLGKMYNIPVYETGVGFKYVAPKMLETNAMIGGEESGGYAFRGNVPERDGILAGLYILDMMVKLQRKPSELIDLLFSKVGPHFYDRIDRTFTGERSAREQAILAANPTTIGGLKVTGLNTTDGFKFSLEDGGWLLIRFSGTEPIMRVYCETTHKDRVPYILKDGLKIAGLE

SEQ ID NO: 8 - protein, 473 aa, Thermanaerothrix daxensis
MGHKIMFGTDGWRGVIAEDYTFDNVRRCAQGFAHYLKTKGYKDEWVVVGYDKRFHSENFAQAAAEVLCGNGFRVYLTDKATPTPVIAYAVVERKAIGAVNITASHNPPTDNGFKVRDASGGAIDPEGLKRIESAIPDEMSAVKRMPASEAEAQGRLVRFDPAPAYIEHLKSLIDLQPIRDAGLKIVVDAMWGNGAGWFPRLLAGGKTEVYEIHNTRNPIFPEMKRPEPIPPNIDVGLRTTVERRADVLVVTDGDADRVGIGDEHGRFVNQLQVYGLLAFYLLEVRGERGPIIKTLSTTSMLEKLGEIYGVPVYETGVGFKYVAPKFLETNALIGGEESGGYAFRGNVPERDGILAGLYFLDMMVRLNRKPSQLLELLFSKVGPHYYDRVDRQFTGDRKTREEMILNANPHTIGGLKVVGLNTLDGFKFLLEDGGWMLIRFSGTEPIIRVYCETTHPDRVQPILQDGLRIAGLA

SEQ ID NO: 9 - protein, 822 aa, Thermotoga maritima
MLEKLPENLKELESLAYNLWWSWSRPAQRLWRMIDSEKWEEHRNPVKILREVSKERLEELSKDEDFIALYELTLERFTDYMEREDTWFNVNYPEWDEKIVYMCMEYGLTKALPIYSGGLGILAGDHLKSASDLGLPLIAVGLLYKHGYFTQQIDSDGRQIEIFPEYDIEELPMKPLRDEDGNQVIVEVPIDNDTVKARVFEVQVGRVKLYLLDTDFEENEDRFRKICDYLYNPEPDVRVSQEILLGIGGMKLLKTLKIKPGVIHLNEGHPAFSSLERIKSYMEEGYSFTEALEIVRQTTVFTTHTPVPAGHDRFPFDFVEKKLTKFFEGFESKELLMNLGKDEDGNFNMTYLALRTSSFINGVSKLHADVSRRMFKNVWKGVPVEEIPIEGITNGVHMGTWINREMRKLFDRYLGRVWREHTDLEGIWYGVDRIPDEELWEAHLNAKKRFIDYIRESIKRRNERLGINEPLPEISENVLIIGFARRFATYKRAVLLFSDLERLKRIVNNSERPVYIVYAGKAHPRDEGGKEFLRRIYEVSQMPDFKNKIIVLENYDIGMARLMVSGVDVWLNNPRRPMEASGTSGMKAAANGVLNASVYDGWWVEGYNGRNGWVIGDESVLPETEADDPKDAEALYELLENEIIPTYYENREKWIFMMKESIKSVAPKFSTTRMLKEYTEKFYIKGLVNREWLERRENVEKIGAWKERILKNWENVSIERIVLEDSKSVEVTVKLGDLTPNDVIVELVAGRGEGMEDLEVWKVIHIRRYRKENDLFVYTYTNGVLGHLGSPGWFYAVRVIPYHPRLPIKFLPEVPVVWKKVL

SEQ ID NO: 10 - protein, 819 aa, Thermus thermophilus
  misc_feature (745)..(745): Xaa can be any naturally occurring amino acid
MNVLGRITAMPDLPEPLEGLKEIAYNLWWSWNPEAAELFQELDPALWKRFRGNPVKLLLELDPARLEALSASGYAARVQATREALRAYLEARRTKRGPLVAYFSAEYGFHSSLPIYAGGLGVLAGDHVKAASDLGLNLVGVGLFYHEGYFHQRLSPEGEQVEVYEPLRPEELPLVPVQDAEGRPVRVAVEFPGRLVHVGGYRVQVGAVPVYLLTTDLPENAPEDRQITARLYAAGLEARIQQELVLGLGGVRFLRALGLAPAFFHMNEGHSAFLGLERLRELVAEGYPFREALELARASALFTTHTPVPAGHDVFPLDLVDRYLGGFWEKLGVDRDTFLGLGLEEKPWGPVFSMSNLALRTAAQANGVSRLHGEVSRNMFRHLWPGLLAEEVPIGHVTNGVHTWTFLHPRLRRHYAEVFGPEWVERPEDPETWRVEGLGEAFWRIRQDLKLFLVREVRQRLYEQRRRNGEGPARLREAEKALDPEALTIGFARRFATYKRAVLLFKDPERLLRILKGPYPVQFVFAGKAHPKDEAGKAYLQELVSKIREYGLEDRMVVLEDYDMYLARVLTHGSDVWLNTPRRPMEASGTSGMKAALNGALNLSVLDGWWAEAYNGKNGFAIGDERVYESEEAQDVADAQALYDLLESEVIPLFYAKGLEGYSSGWMSMVHESLRTVGPYFSAGRMVRDYLALYERGALWEKEARARLEALKAFAEALPAFHALGVRPEVPGDLTLNGGRLEVGXVLEGEVPEGLRPHLRVQLVVRRLGGGLEVVDLEEVAPGRYRTAFRPTRPGSYTYGLRLALLHPVTGRVEWVRWA

SEQ ID NO: 11 - protein, 809 aa, Thermus sp. CCB_US3_UF1
MPLLPEPLSGLKELAYNLWWSWNPEAAELFQEIDPSLWKRFRGNPVKLLLEADPGRLEGLAATSYPARVGAVVEALRAYLREREEKQGPLVAYFSAEYGFHSSLPIYSGGLGVLAGDHVKAASDLGLNLVGVGIFYHEGYFHQRLSPEGVQVEVYETLHPEELPLYPVQDREGRPLRVGVEFPGRTLWLSAYRVQVGAVPVYLLTANLPENTPEDRAITARLYAPGLEMRIQQELVLGLGGVRLLRALGLAPEVFHMNEGHSAFLGLERVRELVAEGHPFPVALELARAGALFTTHTPVPAGHDAFPLELVERYLGGFWERMGTDRETFLSLGLEEKPWGKVFSMSNLALRTSAQANGVSRLHGEVSREMFHHLWPGFLREEVPIGHVTNGVHTWTFLHPRLRRHYAEVFGPEWRKRPEDPETWKVEALGEEFWQIHKDLRAELVREVRTRLYEQRRRNGESPSRLREAEKVLDPEALTIGFARRFATYKRAVLLFKDPERLRRLLHGHYPIQFVFAGKAHPKDEPGKAYLQELFAKIREYGLEDRMVVLEDYDMYLARVLVHGSDVWLNTPRRPMEASGTSGMKAALNGALNLSVLDGWWAEAYNGKNGFAIGDERVYESEEAQDMADAQALYDVLEFEVLPLFYAKGPEGYSSGWLSMVHESLRTVGPRYSAARMVGDYLEIYRRGGAWAEAARAGQEALAAFHQALPALQGVTLRAQVPGDLTLNGVPMRVRAFLEGEVPEALRPFLEVQLVVRRSSGHLEVVPMRPGPDGYEVAYRPSRPGSYAYGVRLALRHPITGHVAWVRWA

SEQ ID NO: 12 - protein, 541 aa, Thermoanaerobacter pseudethanolicus strain ATCC 33223
MGNEKLPRVAYFCMEYGLQSDFKLYAGGLGILAGDHLKAAKELGMPLVGIGILWKQGYTEQHIGEDGYPYDAYRNYTRKYDFLKDTGVKVKVKIRNRNVYCKVWLIDNFDNAPLYLLDTDIPENGDRWITGQLYGWFGEERVAQEIVLGIGGVRALRALGIDVDVYHFNEGHAVLAAIELIREKMENQNMSFEEAWKATREEVVFTTHTPVKEGNESHDLELLMYMGANNGLSIEQMAQIGGVPFNMTVAGLRLSRIANGVSKLHGQTANKMWQHVDNKAPIISITNGIDRNTWVDKRIIEAYNKGEGLLETHNILKQELIDFVYQRTGVKLDADKLLIGFSRRAAPYKRSDLIFTNDEVIGDYLRSKKIQMVFSGKGHPLDDVGKKIVAKLIEMTKKYPESVVFLEDYDMTIGKMLTRGTDVWLNNPRRPLEASGTSGMKAAMNGVLNLSILDGWWAEACIDGVNGWQFGDGFESDNIEELDKHDLEALYDVLLNKVVPTYYNDKAKWENMMRESIRTTYEAFSANRMLKEYYDLMYTKK

SEQ ID NO: 13 - protein, 578 aa, Thermanaerovibrio acidaminovorans strain ATCC 49978
MTIMTYGDNIGNSMLKTLEHDPVFRSVAYFSMEIAIRPEIPTYSGGLGVLAGDIIKSAADLGVPMAAVTLLYRKGYFIQHVDQEGYQRESPVEWKPEEYLTLLPNEISVMLEGRPVKVRAWVYDYVGQSGYPLPIYFLDTDFESNAPADRNLTWHLYGGDQRYRLCQELILGVGGLRMLRDLGYRNIKTFHLNEGHAGFITLELLREQGYEDYDKIRDKVIFTTHTPVPAGHDHFSYELIDKVMDPVFVHHIKRMMGPEGVSMTELGLRYSRYTNAVSIKHAEVSRNMFNSANIDAVTNGVHSTTWTCPGFAKLYDRYIAGWRNDPSRLIQALQLPDEEVWKAHQAAKMKLLARVLEETGRELDADVLTIGFARRAAAYKRADLLFSDVKRLIDVCSGQVQFIFAGKAHPHDEPGKAMIKRIHQMAKEIGSAVPIVFLENYDMSLASLLTSGVDLWLNNPRRPREASGTSGMKCTHNGVMNFSVLDGWWIEGWVEDVTGWSIGPDPEEAELVEYDEMQDAMDLYNKLEDKVIPTYYQHREKWIWMMKHAIALNASYFNTHRVVKEYCEKAYGVVFRGL

SEQ ID NO: 14 - protein, 659 aa, Thermococcus litoralis
MERINFIFGIHNHQPLGNFGWVFEEAYNRSYRPFMEILEEFPEMKVNVHFSGPLLEWIEENKPDYLDLLRSLIKRGQLEIVVAGFYEPVLAAIPKEDRLVQIEMLKDYARKLGYDAKGVWLTERVWQPELVKSLREAGIEYVVVDDYHFMSAGLSKEELFWPYYTEDGGEVITVFPIDEKLRYLIPFRPVKKTIEYLESLTSDDPSKVAVFHDDGEKFGVWPGTYEWVYEKGWLREFFDAITSNEKINLMTYSEYLSKFTPRGLVYLPIASYFEMSEWSLPAKQAKLFVEFVEQLKEEGKFEKYRVFVRGGIWKNFFFKYPESNFMHKRMLMVSKAVRDNPEARKYILKAQCNDAYWHGVFGGIYLPHLRRTVWENIIKAQRYLKPENKILDVDFDGRAEIMVENDGFIATIKPHYGGSIFELSSKRKAVNYNDVLPRRWEHYHEVPEATKPEKESEEGIASIHELGKQIPEEIRRELAYDWQLRAILQDHFIKPEETLDNYRLVKYHELGDFVNQPYEYEMIENGVKLWREGGVYAEEKIPARVEKKIELTEDGFIAKYRVLLEKPYKALFGVEINLAVHSVMEKPEEFEAKEFEVNDPYGIGKVRIELDKAAKVWKFPIKTLSQSEAGWDFIQQGVSYTMLFPIEKELEFTVRFREL

SEQ ID NO: 15 - protein, 503 aa, Oceanithermus profundus DSM 14977
MELPRSFGILLHPTSFPGPYPIGNLGDEARSFLDWLAATGARWWQVLPLGPTGFGDSPYQAFSAFAGNPYLIDPRRLVARGWLEAADPPESPPDRVDYGLVYRWIWPLLRRAYAGFRARATREDTHALAVFEREHADWLEDYALFMALKGEHGGAPWWSWPEPLKRRDPGALAAARERLAEEAAFQRWTQWVFFSQWRALANAAHDLGLGIVGDMPIFVAHDSADVWAHPELFQLDEDLNPVAVAGVPPDYFSPTGQLWGNPLYDWDALERSGFDWWLRRIRRALETADLVRIDHFRGFEAYWAVPAGAPTAEHGRWEKAPGEAFFRKVEATFGSVPILAEDLGLITPEVEALRDRFGLPGMKVLQFAFTGEDNPFLPHNYPESGNCVVYTGTHDNDTTRGWCEHAPDAELDFMRRYLEGRGIACRGCQDAPWALIELALQSRCRMAVFPLQDPLELGSEARMNFPSRPEGNWAWRYSTRDLTHGLAERLRGLAERYARLRRG

SEQ ID NO: 16 - protein, 500 aa, Meiothermus silvanus strain ATCC 700542
MDIPRSFGILLHPTSFPGRWGIGTLGAEARRFVDWLASTGAHWWQVLPLGPTSYGDSPYQSFSAFAGNPYLIDPDILIEKGWLEPEEPPAYPPHKVDYGWLYVTRWDLLRRAYDGFVGRGKPEDLEAFARYRQQEADWLEDYALFMALKHSFGGRPWNEWTAPLRRREPAALEQARKEYADEIGFHAWTQWVFFQQWGDLRNYAHARGIKLIGDMPIFLAYDSSDVWANPQYFYLDAEGLPTVVAGVPPDYFSETGQLWGNPLYRWEVMQAEGFGWWIHRIKKSLEACELVRIDHFRGFEAYWEVPFGEPTAVKGRWVKAPGKELFQAVRAALGDAAIIAEDLGVITPEVEELRDSNGFPGMKILQFAFSDETNPFLPHNYPESGNVIVYTGTHDNDTTIGWYQTAPKEELAFMDKYLEQYGLKIEKPEDAPWVLAELGFRSRAKLVILPLQDVLRLGPEARMNFPGTLGNNWSWRYAPGDLTPELALHLRELARSSDRL

SEQ ID NO: 17 - protein, 511 aa, Anaerolinea thermophila strain DSM 14523
MSLFKRASGILLHPTSLPGPDGIGDLGPEAYRWVNFLAESGCSLWQILPLGPTGFGDSPYQCFSAFAGNPYLVSPALLLDEGLLTSEDLADRPEFPASRVDYGPVIQWKLTLLDRAYVRFKRSTSQKRKAAFEAFKEEQRAWLLDFSLFMAIKEAHGGASWDYWPEPLRKRDPEALNAFHRAHEVDVERHSFRQFLFFRQWQALRQYAHEKGVQIIGDVPIFVAYDSADVWSHPDLFYLDETGKPTVVAGVPPDYFSATGQLWGNPLYRWDYHRETGFAWWLERLKATFAMVDIVRLDHFRGFAGYWEVPYGMPTAEKGRWVPGPGIALFEAIRNALGGLPIIAEDLGEITPDVIELREQLGLPGMKIFQFAFASDADDPFLPHNYVQNCVAYTGTHDNDTAIGWYNSAPEKERDFVRRYLARSGEDIAWDMIRAVWSSVAMFAIAPLQDFLKLGPEARMNYPGRPAGNWGWRYEAFMLDDGLKNRIKEINYLYGRLPEHMKPPKVVKKWT

SEQ ID NO: 18 - protein, 488 aa, Thermoanaerobacterium thermosaccharolyticum
MALKNKVQLITYPDSLGGNLKTLNDVLEKYFSDVFGGVHILPPFPSSGDRGFAPITYSEIEPKFGTWYDIKKMAENFDILLDLMVNHVSRRSIYFQDFLKKGRKSEYADMFITLDKLWKDGKPVKGDIEKMFLRRTLPYSTFKIEETGEEEKVWTTFGKTDPSEQIDLDVNSHLVREFLLEVFKTFSNFGVKIVRLDAVGYVIKKIGTSCFFVEPEIYEFLDWAKGQAASYGIELLLEVHSQFEVQYKLAERGFLIYDFILPFTVLYTLINKSNEMLYHYLKNRPINQFTMLDCHDGIPVKPDLDGLIDTKKAKEVVDICVQRGANLSLIYGDKYKSEDGFDVHQINCTYYSALNCDDDAYLAARAIQFFTPGIPQVYYVGLLAGVNDFEAVKKTKEGREINRHNYGLKEIEESVQKNVVQRLLKLIRFRNEYEAFNGEFFIEDCRKDEIRLTWKKDDKRCSLFIDLKTYKTTIDYINENGEEVKYLV

SEQ ID NO: 19 - protein, 488 aa, Thermoanaerobacterium sp. PSU-2
MALNNKVQLITYPDSLGGDLKTLNDVLGKYFYDVFGGIHILPPFPSSGDRGFAPITYREIEPKFGTWHDIKKMSENFDILLDLMVNHVSRRSIYFQDFLKKGRKSEYADMFITLDKLWKDGKPVKTDIEKMFLRRTLPYSTFKIEETGEEEKVWTTFGKTDPSEQIDLDVNSHLAKEFLLGVFKTFSNFGVNIVRLDAVGYVIKKIGTSCFFVEPEIYEFLNWIKGQAASYGIELLLEVHSQFEIQYKLAERDFWIYDFILPFTVLYTLINKSNEMLYDYLKNRPMNQFTMLDCHDGIPVKPDLDGLIDTKKAKKVVDICVLRGANLSLIYGDKYKSEDGFDVHQINCTYYSALNCDDDAYLAARAIQFFTPGIPQIYYVGLLAGVNDFEAVKRTKEGREINRHNYSLNEIEESVKEDVVQRLLKLIRFRNRYEAFNGEFLVEDCKDDEIRLTWEKDDKRCSLFIDLKTYKTVINYIDENGREVEYVV

SEQ ID NO: 20 - protein, 488 aa, Thermoanaerobacterium thermosaccharolyticum
MALNNKVQLITYPDSLGGDLKTLNDVLEKYFSDVFGGIHILPPFPSSGDRGFAPITYSEIEPKFGTWYDIKKMAENFDILLDLMVNHVSRRSIYFQDFLKKGRKSEYADMFITLDKLWKDGKPVKGDIEKMFLRRTLPYSTFKIEETGEEEKVWTTFGKTDPSEQIDLDVNSHLVKEFLLEVFRTFSNFGVNIVRLDAVGYVIKKIGTSCFFVEPEIYEFLDWAKGQAASYGIELLLEVHSQFEIQYKLAERGFWIYDFILPFTVLYTLINKSNEMLYDYLKNRPINQFTMLDCHDGIPVKPDLDGLIDTKKARDVVDICVQRGANLSLIYGDKYKSEDGFDVHQIGCTYYSALNCDDDAYLAARAIQFFTPGIPQVYYVGLLAGVNDFEAVKKTKEGREINRHNYGLKEIEESVQKKAVQRLLKLIRFRNEYEAFNGEFMVQDCQKDEIRLTWKKDDKRCSLFIDLKTYKTTIDYINENGEEVKYLV

SEQ ID NO: 21 - protein, 488 aa, Thermoanaerobacterium xylanolyticum
MALNNKVQLITYPDSLGGDLKTLNDVLEKYFSDVFGGIHILPPFPSSGDRGFAPITYSEIDPKFGSWYDIKKMADNFDILLDLMVNHVSRRSIYFQDFLKKGRMSEYADMFITLDKLWKDGKPVKTDIEKMFLRRTLPYSTFKIEETGEEERVWTTFGKTDPSEQIDLDVNSHLVREFLLEVFKTFSNFGVNIVRLDAVGYVIKKMGTSCFFVEPDIYEFLNWIKGQAASYGIELLLEVHSQFEVQYKLAERGFWIYDFILPFTVLYTLINRSNEMLYDYLKNRPMNQFTMLDCHDGIPVKPDLDGLIDTKKAKEVVDICVQRGANLSLIYGDKYKSEDGFDVHQIGCTYYSALNCDDDAYLAARAIQFFTPGIPQVYYVGLLAGVNDFEAVKRTKEGREINRHNYGLNEIEESVQKDVVQRLLKLIRFRNRYEAFNGEFLVEDCKDDEIRLTWEKDDKHCSLFIDLGSYRTIVNYVDENGKDVEYIV

SEQ ID NO: 22 - protein, 488 aa, Thermobacillus sp. ZCTH02-B1
MKLENRVQLITYPDSLGGNLAALREVLRRHFPGLFLGGIHILPPFPSSGDRGFAPLDYGMIDPAFGTWEDIAQLGEEYGVMLDVMVNHISRRSPQFMDFLKQGRSSPYADMFLTLDKIWPDGRPVQADIDKMFLRRKLPYSAFTVGDGREELVWTTFGKTDPSEQIDLDVRSPLARHYLSGIFQRFKANRVNMVRLDAVGYVIKKPGTSCFFVEPDIYEFLDWVADQAKEHDIALLPEVHAHYSIQYKLAERGFWIYDFILPFMVLDALVNRSSAMLLRYLRTRPANQFTMLDCHDGIPVKPDLDDLVDTAQARRVVDLCLARGANLSYVISDRHKSPDGFDVHQIRCTYYDALGRNDDAYLAARAIQLFVPGIPQIYYVGLLAGENDPARAEATGDGREINRHNYTLEEIEQAVRRPVVQRLLKLIRFRNEHEAFQGSFRVCESEDSKIRLEWEKDAIRCALHVDLDTYRSIITCTDGQGKEAQWVV

SEQ ID NO: 23 - protein, 504 aa, Bifidobacterium adolescentis [sequence omitted]

SEQ ID NO: 24 - protein, 480 aa, Paenibacillus thermophilus
MKIKNEAMLITYADSLGTNLKELNQVLDKHLQGVVGGVHLLPFYPSSGDRGFAPMDYTKVDPAFGDWSDVEQMSQKYYMMYDFMINHISRQSPYFQDFLENKDESAYKDLFIRYKNFWPGGEPTPEDVDLIYKRKPRAPYVEVTFKDGSTEKVWCTFDEQQIDLDVTTDTTKKFIRDNLTFLAQKGASIIRLDAFAYANKKIGTNCFFVEPDIWDMLRYSKDIISPSGITVLPEIHEHYSIQLKIAEQDYYVYDFALPMLVLHALYSGQVHRLVHWLNICPRKQFTTLDTHDGIGVVDVKDLLSDEECEMTRESLYSQGANVKKIYSTEAYNNLDIYQINCTYYSALGNNDQSYLLARAIQCFAPGIPQIYYVGLLAGENDIELLERTKEGRNINRHYYTLEEIEREVERPVVKQLFRLLKFRNTCPAFDGTVEAEQADINNLRIIWKNGASEAKLEANLATKEFSIRYKDAETNWTLLM

SEQ ID NO: 25 - protein, 489 aa, Tepidibacillus decaturensis
MNVKNQVQLITYPDSLGGNLKNLHHVLLKYFVDIFKGGVHILPPYPSSGDRGFAPINYLEIDPRFGTWADIKAIGENFDVMLDLMVNHISRQSLYFQDFLKKGRQSEYADMFITLDKIWDDGEPVQEDIDKMFLRRPLPYSTFSIKETGEQERVWTTFGKTDPSEQIDLDIKSQKVKQLLTSFFQNFKQQNVKMVRLDAVGYVIKKLGTSCFFVEPDIYDFLDWMREIADSMEIELLPEVHAHYSIQYKLAEHGFWIYDFILPYRILDALVNKSSKDLLDYLKNRPHKQVTMLDCHDGIPVKPDLDDLIDTKEARKLVNVCLERGSNLSLILSHEHKDKDGFDVHQIRCSYYSVLNRDDDAYLAARAIQFFTPGIPQVYYVGLLAGENDMEGVKKTGEGREINRHNFSLDEIEHSLNKKVVQRLLQLIRFRNEYDAFNGEFKVLDSAQDEIRLSWQKEEKRCTLQIDLKTNKSVIEYVDEKDGEIPYFI

SEQ ID NO: 26 - protein, 504 aa, Thermanaerothrix daxensis
MKNQVQLITYVDRLGSGNIKTLHQLLRGPLAGLFGGVHLLPFYYPIKGADAGFDPIDHTRVDPCLGSWEDIRALGQDVDLMADLIVNHISSSSPQFLDYLEKGDDSIYKDLFLTMSSVFPNGATEADLLTIYRPRPGLPFSYITLKNGQKRLLWTTFSRQQIDINVLHPMGREYLHSVLRTLHENGIRMVRLDAVGYAVKKAGTTCFMIPETFDFIENLTHQAQELGMEVLVEIHSHYRKQIEIARQVDRVYDFALPPLVLHAIFNRTAYYLKQWLSISPRNAITVLDTHDGIGVIDIGADSSDPQNYPGLIPPEELEALVEQIHLNSNGQSRLASGAAASNLDLYQVNCTFYDALGRNDRDYLLARAIQFFSPGIPQVYYVGLLAGENDMDLLARTGVGRDINRHYYTLEEIAQAIQRPVVQSLFRLIRFRNQHPAFNGAFSMPESPDSRLILRWDNGAAWAVLEVDFAAGTFSISGSPLEGAEPIEALPGAHPDNRYGGIAT